European Patent Application EP 4 286 521 A1, published December 6, 2023. Title: GENE THERAPIES FOR TREATING NEURODEGENERATIVE DISORDER. Applicant: ABrain. The sequence listing filed with the application follows.

SEQUENCE LISTING (72 sequences)

SEQ ID NO: 1 - protein, 770 aa, Artificial Sequence
  amyloid precursor protein
MLPGLALLLLAAWTARALEVPTDGNAGLLAEPQIAMFCGRLNMHMNVQNGKWDSDPSGTKTCIDTKEGILQYCQEVYPELQITNVVEANQPVTIQNWCKRGRKQCKTHPHFVIPYRCLVGEFVSDALLVPDKCKFLHQERMDVCETHLHWHTVAKETCSEKSTNLHDYGMLLPCGIDKFRGVEFVCCPLAEESDNVDSADAEEDDSDVWWGGADTDYADGSEDKVVEVAEEEEVAEVEEEEADDDEDDEDGDEVEEEAEEPYEEATERTTSIATTTTTTTESVEEVVREVCSEQAETGPCRAMISRWYFDVTEGKCAPFFYGGCGGNRNNFDTEEYCMAVCGSAMSQSLLKTTQEPLARDPVKLPTTAASTPDAVDKYLETPGDENEHAHFQKAKERLEAKHRERMSQVMREWEEAERQAKNLPKADKKAVIQHFQEKVESLEQEAANERQQLVETHMARVEAMLNDRRRLALENYITALQAVPPRPRHVFNMLKKYVRAEQKDRQHTLKHFEHVRMVDPKKAAQIRSQVMTHLRVIYERMNQSLSLLYNVPAVAEEIQDEVDELLQKEQNYSDDVLANMISEPRISYGNDALMPSLTETKTTVELLPVNGEFSLDDLQPWHSFGADSVPANTENEVEPVDARPAADRGLTTRPGSGLTNIKTEEISEVKMDAEFRHDSGYEVHHQKLVFFAEDVGSNKGAIIGLMVGGVVIATVIVITLVMLKKKQYTSIHHGVVEVDAAVTPEERHLSKMQQNGYENPTYKFFEQMQN

SEQ ID NO: 2 - DNA, 2313 bp, Artificial Sequence
  amyloid precursor protein
atgctgcccggtttggcactgctcctgctggccgcctggacggctcgggcgctggaggtacccactgatggtaatgctggcctgctggctgaaccccagattgccatgttctgtggcagactgaacatgcacatgaatgtccagaatgggaagtgggattcagatccatcagggaccaaaacctgcattgataccaaggaaggcatcctgcagtattgccaagaagtctaccctgaactgcagatcaccaatgtggtagaagccaaccaaccagtgaccatccagaactggtgcaagcggggccgcaagcagtgcaagacccatccccactttgtgattccctaccgctgcttagttggtgagtttgtaagtgatgcccttctcgttcctgacaagtgcaaattcttacaccaggagaggatggatgtttgcgaaactcatcttcactggcacaccgtcgccaaagagacatgcagtgagaagagtaccaacttgcatgactacggcatgttgctgccctgcggaattgacaagttccgaggggtagagtttgtgtgttgcccactggctgaagaaagtgacaatgtggattctgctgatgcggaggaggatgactcggatgtctggtggggcggagcagacacagactatgcagatgggagtgaagacaaagtagtagaagtagcagaggaggaagaagtggctgaggtggaagaagaagaagccgatgatgacgaggacgatgaggatggtgatgaggtagaggaagaggctgaggaaccctacgaagaagccacagagagaaccaccagcattgccaccaccaccaccaccaccacagagtctgtggaagaggtggttcgagaggtgtgctctgaacaagccgagacggggccgtgccgagcaatgatctcccgctggtactttgatgtgactgaagggaagtgtgccccattcttttacggcggatgtggcggcaaccggaacaactttgacacagaagagtactgcatggccgtgtgtggcagcgccatgtcccaaagtttactcaagactacccaggaacctcttgcccgagatcctgttaaacttcctacaacagcagccagtacccctgatgccgttgacaagtatctcgagacacctggggatgagaatgaacatgcccatttccagaaagccaaagagaggcttgaggccaagcaccgagagagaatgtcccaggtcatgagagaatgggaagaggcagaacgtcaagcaaagaacttgcctaaagctgataagaaggcagttatccagcatttccaggagaaagtggaatctttggaacaggaagcagccaacgagagacagcagctggtggagacacacatggccagagtggaagccatgctcaatgaccgccgccgcctggccctggagaactacatcaccgctctgcaggctgttcctcctcggcctcgtcacgtgttcaatatgctaaagaagtatgtccgcgcagaacagaaggacagacagcacaccctaaagcatttcgagcatgtgcgcatggtggatcccaagaaagccgctcagatccggtcccaggttatgacacacctccgtgtgatttatgagcgcatgaatcagtctctctccctgctctacaacgtgcctgcagtggccgaggagattcaggatgaagttgatgagctgcttcagaaagagcaaaactattcagatgacgtcttggccaacatgattagtgaaccaaggatcagttacggaaacgatgctctcatgccatctttgaccgaaacgaaaaccaccgtggagctccttcccgtgaatggagagttcagcctggacgatctccagccgtggcattcttttggggctgactctgtgccagccaacacagaaaacgaagttgagcctgttgatgcccgccctgctgccgaccgaggactgaccactcgaccaggttctgggttgacaaatatcaagacggaggagatctctgaagtgaagatggatgcagaattccgacatgactcaggatatgaagttcatcatcaaaaattggtgttctttgcagaagatgtgggttcaaacaaaggtgcaatcattggactcatggtgggcggtgttgtcatagcgacagtgatcgtcatcaccttggtgatgctgaagaagaaacagtacacatccattcatcatggtgtggtggaggttgacgccgctgtcaccccagaggagcgccacctgtccaagatgcagcagaacggctacgaaaatccaacctacaagttctttgagcagatgcagaactag

SEQ ID NO: 3 - DNA, 2313 bp, Artificial Sequence
  amyloid precursor protein  F690D/L705P
atgctgcccggtttggcactgctcctgctggccgcctggacggctcgggcgctggaggtacccactgatggtaatgctggcctgctggctgaaccccagattgccatgttctgtggcagactgaacatgcacatgaatgtccagaatgggaagtgggattcagatccatcagggaccaaaacctgcattgataccaaggaaggcatcctgcagtattgccaagaagtctaccctgaactgcagatcaccaatgtggtagaagccaaccaaccagtgaccatccagaactggtgcaagcggggccgcaagcagtgcaagacccatccccactttgtgattccctaccgctgcttagttggtgagtttgtaagtgatgcccttctcgttcctgacaagtgcaaattcttacaccaggagaggatggatgtttgcgaaactcatcttcactggcacaccgtcgccaaagagacatgcagtgagaagagtaccaacttgcatgactacggcatgttgctgccctgcggaattgacaagttccgaggggtagagtttgtgtgttgcccactggctgaagaaagtgacaatgtggattctgctgatgcggaggaggatgactcggatgtctggtggggcggagcagacacagactatgcagatgggagtgaagacaaagtagtagaagtagcagaggaggaagaagtggctgaggtggaagaagaagaagccgatgatgacgaggacgatgaggatggtgatgaggtagaggaagaggctgaggaaccctacgaagaagccacagagagaaccaccagcattgccaccaccaccaccaccaccacagagtctgtggaagaggtggttcgagaggtgtgctctgaacaagccgagacggggccgtgccgagcaatgatctcccgctggtactttgatgtgactgaagggaagtgtgccccattcttttacggcggatgtggcggcaaccggaacaactttgacacagaagagtactgcatggccgtgtgtggcagcgccatgtcccaaagtttactcaagactacccaggaacctcttgcccgagatcctgttaaacttcctacaacagcagccagtacccctgatgccgttgacaagtatctcgagacacctggggatgagaatgaacatgcccatttccagaaagccaaagagaggcttgaggccaagcaccgagagagaatgtcccaggtcatgagagaatgggaagaggcagaacgtcaagcaaagaacttgcctaaagctgataagaaggcagttatccagcatttccaggagaaagtggaatctttggaacaggaagcagccaacgagagacagcagctggtggagacacacatggccagagtggaagccatgctcaatgaccgccgccgcctggccctggagaactacatcaccgctctgcaggctgttcctcctcggcctcgtcacgtgttcaatatgctaaagaagtatgtccgcgcagaacagaaggacagacagcacaccctaaagcatttcgagcatgtgcgcatggtggatcccaagaaagccgctcagatccggtcccaggttatgacacacctccgtgtgatttatgagcgcatgaatcagtctctctccctgctctacaacgtgcctgcagtggccgaggagattcaggatgaagttgatgagctgcttcagaaagagcaaaactattcagatgacgtcttggccaacatgattagtgaaccaaggatcagttacggaaacgatgctctcatgccatctttgaccgaaacgaaaaccaccgtggagctccttcccgtgaatggagagttcagcctggacgatctccagccgtggcattcttttggggctgactctgtgccagccaacacagaaaacgaagttgagcctgttgatgcccgccctgctgccgaccgaggactgaccactcgaccaggttctgggttgacaaatatcaagacggaggagatctctgaagtgaagatggatgcagaattccgacatgactcaggatatgaagttcatcatcaaaaattggtggactttgcagaagatgtgggttcaaacaaaggtgcaatcattggacccatggtgggcggtgttgtcatagcgacagtgatcgtcatcaccttggtgatgctgaagaagaaacagtacacatccattcatcatggtgtggtggaggttgacgccgctgtcaccccagaggagcgccacctgtccaagatgcagcagaacggctacgaaaatccaacctacaagttctttgagcagatgcagaactag

SEQ ID NO: 4 - DNA, 2313 bp, Artificial Sequence
  amyloid precursor protein  F691P
atgctgcccggtttggcactgctcctgctggccgcctggacggctcgggcgctggaggtacccactgatggtaatgctggcctgctggctgaaccccagattgccatgttctgtggcagactgaacatgcacatgaatgtccagaatgggaagtgggattcagatccatcagggaccaaaacctgcattgataccaaggaaggcatcctgcagtattgccaagaagtctaccctgaactgcagatcaccaatgtggtagaagccaaccaaccagtgaccatccagaactggtgcaagcggggccgcaagcagtgcaagacccatccccactttgtgattccctaccgctgcttagttggtgagtttgtaagtgatgcccttctcgttcctgacaagtgcaaattcttacaccaggagaggatggatgtttgcgaaactcatcttcactggcacaccgtcgccaaagagacatgcagtgagaagagtaccaacttgcatgactacggcatgttgctgccctgcggaattgacaagttccgaggggtagagtttgtgtgttgcccactggctgaagaaagtgacaatgtggattctgctgatgcggaggaggatgactcggatgtctggtggggcggagcagacacagactatgcagatgggagtgaagacaaagtagtagaagtagcagaggaggaagaagtggctgaggtggaagaagaagaagccgatgatgacgaggacgatgaggatggtgatgaggtagaggaagaggctgaggaaccctacgaagaagccacagagagaaccaccagcattgccaccaccaccaccaccaccacagagtctgtggaagaggtggttcgagaggtgtgctctgaacaagccgagacggggccgtgccgagcaatgatctcccgctggtactttgatgtgactgaagggaagtgtgccccattcttttacggcggatgtggcggcaaccggaacaactttgacacagaagagtactgcatggccgtgtgtggcagcgccatgtcccaaagtttactcaagactacccaggaacctcttgcccgagatcctgttaaacttcctacaacagcagccagtacccctgatgccgttgacaagtatctcgagacacctggggatgagaatgaacatgcccatttccagaaagccaaagagaggcttgaggccaagcaccgagagagaatgtcccaggtcatgagagaatgggaagaggcagaacgtcaagcaaagaacttgcctaaagctgataagaaggcagttatccagcatttccaggagaaagtggaatctttggaacaggaagcagccaacgagagacagcagctggtggagacacacatggccagagtggaagccatgctcaatgaccgccgccgcctggccctggagaactacatcaccgctctgcaggctgttcctcctcggcctcgtcacgtgttcaatatgctaaagaagtatgtccgcgcagaacagaaggacagacagcacaccctaaagcatttcgagcatgtgcgcatggtggatcccaagaaagccgctcagatccggtcccaggttatgacacacctccgtgtgatttatgagcgcatgaatcagtctctctccctgctctacaacgtgcctgcagtggccgaggagattcaggatgaagttgatgagctgcttcagaaagagcaaaactattcagatgacgtcttggccaacatgattagtgaaccaaggatcagttacggaaacgatgctctcatgccatctttgaccgaaacgaaaaccaccgtggagctccttcccgtgaatggagagttcagcctggacgatctccagccgtggcattcttttggggctgactctgtgccagccaacacagaaaacgaagttgagcctgttgatgcccgccctgctgccgaccgaggactgaccactcgaccaggttctgggttgacaaatatcaagacggaggagatctctgaagtgaagatggatgcagaattccgacatgactcaggatatgaagttcatcatcaaaaattggtgttccctgcagaagatgtgggttcaaacaaaggtgcaatcattggactcatggtgggcggtgttgtcatagcgacagtgatcgtcatcaccttggtgatgctgaagaagaaacagtacacatccattcatcatggtgtggtggaggttgacgccgctgtcaccccagaggagcgccacctgtccaagatgcagcagaacggctacgaaaatccaacctacaagttctttgagcagatgcagaactag

SEQ ID NO: 5 - DNA, 2313 bp, Artificial Sequence
  amyloid precursor protein  V689P/A692D
atgctgcccggtttggcactgctcctgctggccgcctggacggctcgggcgctggaggtacccactgatggtaatgctggcctgctggctgaaccccagattgccatgttctgtggcagactgaacatgcacatgaatgtccagaatgggaagtgggattcagatccatcagggaccaaaacctgcattgataccaaggaaggcatcctgcagtattgccaagaagtctaccctgaactgcagatcaccaatgtggtagaagccaaccaaccagtgaccatccagaactggtgcaagcggggccgcaagcagtgcaagacccatccccactttgtgattccctaccgctgcttagttggtgagtttgtaagtgatgcccttctcgttcctgacaagtgcaaattcttacaccaggagaggatggatgtttgcgaaactcatcttcactggcacaccgtcgccaaagagacatgcagtgagaagagtaccaacttgcatgactacggcatgttgctgccctgcggaattgacaagttccgaggggtagagtttgtgtgttgcccactggctgaagaaagtgacaatgtggattctgctgatgcggaggaggatgactcggatgtctggtggggcggagcagacacagactatgcagatgggagtgaagacaaagtagtagaagtagcagaggaggaagaagtggctgaggtggaagaagaagaagccgatgatgacgaggacgatgaggatggtgatgaggtagaggaagaggctgaggaaccctacgaagaagccacagagagaaccaccagcattgccaccaccaccaccaccaccacagagtctgtggaagaggtggttcgagaggtgtgctctgaacaagccgagacggggccgtgccgagcaatgatctcccgctggtactttgatgtgactgaagggaagtgtgccccattcttttacggcggatgtggcggcaaccggaacaactttgacacagaagagtactgcatggccgtgtgtggcagcgccatgtcccaaagtttactcaagactacccaggaacctcttgcccgagatcctgttaaacttcctacaacagcagccagtacccctgatgccgttgacaagtatctcgagacacctggggatgagaatgaacatgcccatttccagaaagccaaagagaggcttgaggccaagcaccgagagagaatgtcccaggtcatgagagaatgggaagaggcagaacgtcaagcaaagaacttgcctaaagctgataagaaggcagttatccagcatttccaggagaaagtggaatctttggaacaggaagcagccaacgagagacagcagctggtggagacacacatggccagagtggaagccatgctcaatgaccgccgccgcctggccctggagaactacatcaccgctctgcaggctgttcctcctcggcctcgtcacgtgttcaatatgctaaagaagtatgtccgcgcagaacagaaggacagacagcacaccctaaagcatttcgagcatgtgcgcatggtggatcccaagaaagccgctcagatccggtcccaggttatgacacacctccgtgtgatttatgagcgcatgaatcagtctctctccctgctctacaacgtgcctgcagtggccgaggagattcaggatgaagttgatgagctgcttcagaaagagcaaaactattcagatgacgtcttggccaacatgattagtgaaccaaggatcagttacggaaacgatgctctcatgccatctttgaccgaaacgaaaaccaccgtggagctccttcccgtgaatggagagttcagcctggacgatctccagccgtggcattcttttggggctgactctgtgccagccaacacagaaaacgaagttgagcctgttgatgcccgccctgctgccgaccgaggactgaccactcgaccaggttctgggttgacaaatatcaagacggaggagatctctgaagtgaagatggatgcagaattccgacatgactcaggatatgaagttcatcatcaaaaattgccgttctttgacgaagatgtgggttcaaacaaaggtgcaatcattggactcatggtgggcggtgttgtcatagcgacagtgatcgtcatcaccttggtgatgctgaagaagaaacagtacacatccattcatcatggtgtggtggaggttgacgccgctgtcaccccagaggagcgccacctgtccaagatgcagcagaacggctacgaaaatccaacctacaagttctttgagcagatgcagaactag

SEQ ID NO: 6 - DNA, 2313 bp, Artificial Sequence
  amyloid precursor protein  V689P/F690D/A692D
atgctgcccggtttggcactgctcctgctggccgcctggacggctcgggcgctggaggtacccactgatggtaatgctggcctgctggctgaaccccagattgccatgttctgtggcagactgaacatgcacatgaatgtccagaatgggaagtgggattcagatccatcagggaccaaaacctgcattgataccaaggaaggcatcctgcagtattgccaagaagtctaccctgaactgcagatcaccaatgtggtagaagccaaccaaccagtgaccatccagaactggtgcaagcggggccgcaagcagtgcaagacccatccccactttgtgattccctaccgctgcttagttggtgagtttgtaagtgatgcccttctcgttcctgacaagtgcaaattcttacaccaggagaggatggatgtttgcgaaactcatcttcactggcacaccgtcgccaaagagacatgcagtgagaagagtaccaacttgcatgactacggcatgttgctgccctgcggaattgacaagttccgaggggtagagtttgtgtgttgcccactggctgaagaaagtgacaatgtggattctgctgatgcggaggaggatgactcggatgtctggtggggcggagcagacacagactatgcagatgggagtgaagacaaagtagtagaagtagcagaggaggaagaagtggctgaggtggaagaagaagaagccgatgatgacgaggacgatgaggatggtgatgaggtagaggaagaggctgaggaaccctacgaagaagccacagagagaaccaccagcattgccaccaccaccaccaccaccacagagtctgtggaagaggtggttcgagaggtgtgctctgaacaagccgagacggggccgtgccgagcaatgatctcccgctggtactttgatgtgactgaagggaagtgtgccccattcttttacggcggatgtggcggcaaccggaacaactttgacacagaagagtactgcatggccgtgtgtggcagcgccatgtcccaaagtttactcaagactacccaggaacctcttgcccgagatcctgttaaacttcctacaacagcagccagtacccctgatgccgttgacaagtatctcgagacacctggggatgagaatgaacatgcccatttccagaaagccaaagagaggcttgaggccaagcaccgagagagaatgtcccaggtcatgagagaatgggaagaggcagaacgtcaagcaaagaacttgcctaaagctgataagaaggcagttatccagcatttccaggagaaagtggaatctttggaacaggaagcagccaacgagagacagcagctggtggagacacacatggccagagtggaagccatgctcaatgaccgccgccgcctggccctggagaactacatcaccgctctgcaggctgttcctcctcggcctcgtcacgtgttcaatatgctaaagaagtatgtccgcgcagaacagaaggacagacagcacaccctaaagcatttcgagcatgtgcgcatggtggatcccaagaaagccgctcagatccggtcccaggttatgacacacctccgtgtgatttatgagcgcatgaatcagtctctctccctgctctacaacgtgcctgcagtggccgaggagattcaggatgaagttgatgagctgcttcagaaagagcaaaactattcagatgacgtcttggccaacatgattagtgaaccaaggatcagttacggaaacgatgctctcatgccatctttgaccgaaacgaaaaccaccgtggagctccttcccgtgaatggagagttcagcctggacgatctccagccgtggcattcttttggggctgactctgtgccagccaacacagaaaacgaagttgagcctgttgatgcccgccctgctgccgaccgaggactgaccactcgaccaggttctgggttgacaaatatcaagacggaggagatctctgaagtgaagatggatgcagaattccgacatgactcaggatatgaagttcatcatcaaaaattgccggactttgacgaagatgtgggttcaaacaaaggtgcaatcattggactcatggtgggcggtgttgtcatagcgacagtgatcgtcatcaccttggtgatgctgaagaagaaacagtacacatccattcatcatggtgtggtggaggttgacgccgctgtcaccccagaggagcgccacctgtccaagatgcagcagaacggctacgaaaatccaacctacaagttctttgagcagatgcagaactag

SEQ ID NO: 7 - protein, 770 aa, Artificial Sequence
  amyloid precursor protein  F690D/L705P
MLPGLALLLLAAWTARALEVPTDGNAGLLAEPQIAMFCGRLNMHMNVQNGKWDSDPSGTKTCIDTKEGILQYCQEVYPELQITNVVEANQPVTIQNWCKRGRKQCKTHPHFVIPYRCLVGEFVSDALLVPDKCKFLHQERMDVCETHLHWHTVAKETCSEKSTNLHDYGMLLPCGIDKFRGVEFVCCPLAEESDNVDSADAEEDDSDVWWGGADTDYADGSEDKVVEVAEEEEVAEVEEEEADDDEDDEDGDEVEEEAEEPYEEATERTTSIATTTTTTTESVEEVVREVCSEQAETGPCRAMISRWYFDVTEGKCAPFFYGGCGGNRNNFDTEEYCMAVCGSAMSQSLLKTTQEPLARDPVKLPTTAASTPDAVDKYLETPGDENEHAHFQKAKERLEAKHRERMSQVMREWEEAERQAKNLPKADKKAVIQHFQEKVESLEQEAANERQQLVETHMARVEAMLNDRRRLALENYITALQAVPPRPRHVFNMLKKYVRAEQKDRQHTLKHFEHVRMVDPKKAAQIRSQVMTHLRVIYERMNQSLSLLYNVPAVAEEIQDEVDELLQKEQNYSDDVLANMISEPRISYGNDALMPSLTETKTTVELLPVNGEFSLDDLQPWHSFGADSVPANTENEVEPVDARPAADRGLTTRPGSGLTNIKTEEISEVKMDAEFRHDSGYEVHHQKLVDFAEDVGSNKGAIIGPMVGGVVIATVIVITLVMLKKKQYTSIHHGVVEVDAAVTPEERHLSKMQQNGYENPTYKFFEQMQN

SEQ ID NO: 8 - protein, 770 aa, Artificial Sequence
  amyloid precursor protein  F691P
MLPGLALLLLAAWTARALEVPTDGNAGLLAEPQIAMFCGRLNMHMNVQNGKWDSDPSGTKTCIDTKEGILQYCQEVYPELQITNVVEANQPVTIQNWCKRGRKQCKTHPHFVIPYRCLVGEFVSDALLVPDKCKFLHQERMDVCETHLHWHTVAKETCSEKSTNLHDYGMLLPCGIDKFRGVEFVCCPLAEESDNVDSADAEEDDSDVWWGGADTDYADGSEDKVVEVAEEEEVAEVEEEEADDDEDDEDGDEVEEEAEEPYEEATERTTSIATTTTTTTESVEEVVREVCSEQAETGPCRAMISRWYFDVTEGKCAPFFYGGCGGNRNNFDTEEYCMAVCGSAMSQSLLKTTQEPLARDPVKLPTTAASTPDAVDKYLETPGDENEHAHFQKAKERLEAKHRERMSQVMREWEEAERQAKNLPKADKKAVIQHFQEKVESLEQEAANERQQLVETHMARVEAMLNDRRRLALENYITALQAVPPRPRHVFNMLKKYVRAEQKDRQHTLKHFEHVRMVDPKKAAQIRSQVMTHLRVIYERMNQSLSLLYNVPAVAEEIQDEVDELLQKEQNYSDDVLANMISEPRISYGNDALMPSLTETKTTVELLPVNGEFSLDDLQPWHSFGADSVPANTENEVEPVDARPAADRGLTTRPGSGLTNIKTEEISEVKMDAEFRHDSGYEVHHQKLVFPAEDVGSNKGAIIGLMVGGVVIATVIVITLVMLKKKQYTSIHHGVVEVDAAVTPEERHLSKMQQNGYENPTYKFFEQMQN

SEQ ID NO: 9 - protein, 770 aa, Artificial Sequence
  amyloid precursor protein  V689P/A692D
MLPGLALLLLAAWTARALEVPTDGNAGLLAEPQIAMFCGRLNMHMNVQNGKWDSDPSGTKTCIDTKEGILQYCQEVYPELQITNVVEANQPVTIQNWCKRGRKQCKTHPHFVIPYRCLVGEFVSDALLVPDKCKFLHQERMDVCETHLHWHTVAKETCSEKSTNLHDYGMLLPCGIDKFRGVEFVCCPLAEESDNVDSADAEEDDSDVWWGGADTDYADGSEDKVVEVAEEEEVAEVEEEEADDDEDDEDGDEVEEEAEEPYEEATERTTSIATTTTTTTESVEEVVREVCSEQAETGPCRAMISRWYFDVTEGKCAPFFYGGCGGNRNNFDTEEYCMAVCGSAMSQSLLKTTQEPLARDPVKLPTTAASTPDAVDKYLETPGDENEHAHFQKAKERLEAKHRERMSQVMREWEEAERQAKNLPKADKKAVIQHFQEKVESLEQEAANERQQLVETHMARVEAMLNDRRRLALENYITALQAVPPRPRHVFNMLKKYVRAEQKDRQHTLKHFEHVRMVDPKKAAQIRSQVMTHLRVIYERMNQSLSLLYNVPAVAEEIQDEVDELLQKEQNYSDDVLANMISEPRISYGNDALMPSLTETKTTVELLPVNGEFSLDDLQPWHSFGADSVPANTENEVEPVDARPAADRGLTTRPGSGLTNIKTEEISEVKMDAEFRHDSGYEVHHQKLPFFDEDVGSNKGAIIGLMVGGVVIATVIVITLVMLKKKQYTSIHHGVVEVDAAVTPEERHLSKMQQNGYENPTYKFFEQMQN

SEQ ID NO: 10 - protein, 770 aa, Artificial Sequence
  amyloid precursor protein V689P/F690D/A692D
MLPGLALLLLAAWTARALEVPTDGNAGLLAEPQIAMFCGRLNMHMNVQNGKWDSDPSGTKTCIDTKEGILQYCQEVYPELQITNVVEANQPVTIQNWCKRGRKQCKTHPHFVIPYRCLVGEFVSDALLVPDKCKFLHQERMDVCETHLHWHTVAKETCSEKSTNLHDYGMLLPCGIDKFRGVEFVCCPLAEESDNVDSADAEEDDSDVWWGGADTDYADGSEDKVVEVAEEEEVAEVEEEEADDDEDDEDGDEVEEEAEEPYEEATERTTSIATTTTTTTESVEEVVREVCSEQAETGPCRAMISRWYFDVTEGKCAPFFYGGCGGNRNNFDTEEYCMAVCGSAMSQSLLKTTQEPLARDPVKLPTTAASTPDAVDKYLETPGDENEHAHFQKAKERLEAKHRERMSQVMREWEEAERQAKNLPKADKKAVIQHFQEKVESLEQEAANERQQLVETHMARVEAMLNDRRRLALENYITALQAVPPRPRHVFNMLKKYVRAEQKDRQHTLKHFEHVRMVDPKKAAQIRSQVMTHLRVIYERMNQSLSLLYNVPAVAEEIQDEVDELLQKEQNYSDDVLANMISEPRISYGNDALMPSLTETKTTVELLPVNGEFSLDDLQPWHSFGADSVPANTENEVEPVDARPAADRGLTTRPGSGLTNIKTEEISEVKMDAEFRHDSGYEVHHQKLPDFDEDVGSNKGAIIGLMVGGVVIATVIVITLVMLKKKQYTSIHHGVVEVDAAVTPEERHLSKMQQNGYENPTYKFFEQMQN

SEQ ID NO: 11 - protein, 42 aa, Artificial Sequence [sequence omitted]

SEQ ID NO: 12 - DNA, 126 bp, Artificial Sequence
  Amyloid beta 42
gatgcagaattccgacatgactcaggatatgaagttcatcatcaaaaattggtgttctttgcagaagatgtgggttcaaacaaaggtgcaatcattggactcatggtgggcggtgttgtcatagcg

SEQ ID NO: 13 - DNA, 126 bp, Artificial Sequence
  Amyloid beta 42 (F19D/L34P)
gatgcagaattccgacatgactcaggatatgaagttcatcatcaaaaattggtggactttgcagaagatgtgggttcaaacaaaggtgcaatcattggacccatggtgggcggtgttgtcatagcg

SEQ ID NO: 14 - DNA, 126 bp, Artificial Sequence
  Amyloid beta 42 (F20P)
gatgcagaattccgacatgactcaggatatgaagttcatcatcaaaaattggtgttccctgcagaagatgtgggttcaaacaaaggtgcaatcattggactcatggtgggcggtgttgtcatagcg

SEQ ID NO: 15 - DNA, 126 bp, Artificial Sequence
  Amyloid beta 42 (V18P/A21D)
gatgcagaattccgacatgactcaggatatgaagttcatcatcaaaaattgccgttctttgacgaagatgtgggttcaaacaaaggtgcaatcattggactcatggtgggcggtgttgtcatagcg

SEQ ID NO: 16 - DNA, 126 bp, Artificial Sequence
  Amyloid beta 42 (V18P/F19D/A21D)
gatgcagaattccgacatgactcaggatatgaagttcatcatcaaaaattgccggactttgacgaagatgtgggttcaaacaaaggtgcaatcattggactcatggtgggcggtgttgtcatagcg

SEQ ID NO: 17 - protein, 42 aa, Artificial Sequence
  Amyloid beta 42 (F19D/L34P)
DAEFRHDSGYEVHHQKLVDFAEDVGSNKGAIIGPMVGGVVIA

SEQ ID NO: 18 - protein, 42 aa, Artificial Sequence
  Amyloid beta 42 (F20P)
DAEFRHDSGYEVHHQKLVFPAEDVGSNKGAIIGLMVGGVVIA

SEQ ID NO: 19 - protein, 42 aa, Artificial Sequence
  Amyloid beta 42 (V18P/A21D)
DAEFRHDSGYEVHHQKLPFFDEDVGSNKGAIIGLMVGGVVIA

SEQ ID NO: 20 - protein, 42 aa, Artificial Sequence
  Amyloid beta 42 (V18P/F19D/A21D)
DAEFRHDSGYEVHHQKLPDFDEDVGSNKGAIIGLMVGGVVIA

SEQ ID NO: 21 - protein, 11 aa, Artificial Sequence
  Tau inhibitor
MDVWMINKKRK

SEQ ID NO: 22 - protein, 11 aa, Artificial Sequence
  Tau inhibitor
MDVQMINKKLK

SEQ ID NO: 23 - protein, 8 aa, Artificial Sequence
  Tau inhibitor
MSVWIWYE

SEQ ID NO: 24 - protein, 11 aa, Artificial Sequence
  Tau inhibitor
MDVQMINKKRK

SEQ ID NO: 25 - protein, 11 aa, Artificial Sequence
  Tau inhibitor
MDVQWINKKRK

SEQ ID NO: 26 - protein, 11 aa, Artificial Sequence
  Tau inhibitor
MDVQRINKKRK

SEQ ID NO: 27 - protein, 11 aa, Artificial Sequence
  Tau inhibitor
MDVWWINKKRK

SEQ ID NO: 28 - protein, 11 aa, Artificial Sequence
  Tau inhibitor
MDVWMWNKKRK

SEQ ID NO: 29 - protein, 11 aa, Artificial Sequence
  Tau inhibitor
MDVWWWNKKRK

SEQ ID NO: 30 - protein, 7 aa, Artificial Sequence
  Tau inhibitor
MVQIVYK

SEQ ID NO: 31 - protein, 21 aa, Artificial Sequence
  Tau inhibitor
TVIVITLVMLKDVWMINKKRK

SEQ ID NO: 32 - protein, 21 aa, Artificial Sequence
  Tau inhibitor
TVIVITLVMLKDVQMINKKLK

SEQ ID NO: 33 - protein, 130 aa, Artificial Sequence
  Tau inhibitor
MQTAPVPMPDLKNVKSKIGSTENLKHQPGGGDVQPINKKLKLSNVQSKCGSKDNIKHVPGGGSVQPVYDPVDLSKVTSKCGSLGNIHHKPGGGQVEVKSEKLDFKDRVQSKIGSLDNITHVPGGGNKKIE

SEQ ID NO: 34 - DNA, 33 bp, Artificial Sequence
  Tau inhibitor
atggacgtatggatgattaacaaaaagagaaag

SEQ ID NO: 35 - DNA, 33 bp, Artificial Sequence
  Tau inhibitor
atggacgtacagatgattaacaaaaagctgaag

SEQ ID NO: 36 - DNA, 24 bp, Artificial Sequence
  Tau inhibitor
atgtccgtgtggatctggtacgag

SEQ ID NO: 37 - DNA, 33 bp, Artificial Sequence
  Tau inhibitor
atggacgtacagatgattaacaaaaagagaaag

SEQ ID NO: 38 - DNA, 33 bp, Artificial Sequence
  Tau inhibitor
atggacgtacagtggattaacaaaaagagaaag

SEQ ID NO: 39 - DNA, 33 bp, Artificial Sequence
  Tau inhibitor
atggacgtacagcggattaacaaaaagagaaag

SEQ ID NO: 40 - DNA, 33 bp, Artificial Sequence
  Tau inhibitor
atggacgtatggtggattaacaaaaagagaaag

SEQ ID NO: 41 - DNA, 33 bp, Artificial Sequence
  Tau inhibitor
atggacgtatggatgtggaacaaaaagagaaag

SEQ ID NO: 42 - DNA, 33 bp, Artificial Sequence
  Tau inhibitor
atggacgtatggtggtggaacaaaaagagaaag

SEQ ID NO: 43 - DNA, 21 bp, Artificial Sequence
  Tau inhibitor
atggtacagattgtgtacaag

SEQ ID NO: 44 - DNA, 63 bp, Artificial Sequence
  Tau inhibitor
acagtgatcgtcatcaccttggtgatgctgaaggacgtatggatgattaacaaaaagagaaag

SEQ ID NO: 45 - DNA, 63 bp, Artificial Sequence
  Tau inhibitor
acagtgatcgtcatcaccttggtgatgctgaaggacgtacagatgattaacaaaaagctgaag

SEQ ID NO: 46 - DNA, 393 bp, Artificial Sequence
  Tau inhibitor
atgcagacagcccccgtgcccatgccagacctgaaaaatgtcaagtccaagatcggctccactgagaacctgaagcaccagccgggaggcggggacgtgcagccaattaataagaagctgaagcttagcaacgtccagtccaagtgtggctcaaaggataatatcaaacacgtcccgggaggcggcagtgtgcaaccagtctacgacccagttgacctgagcaaggtgacctccaagtgtggctcattaggcaacatccatcataaaccaggaggtggccaggtggaagtaaaatctgagaagcttgacttcaaggacagagtccagtcgaagattgggtccctggacaatatcacccacgtccctggcggaggaaataaaaagattgaatga

SEQ ID NO: 47 - protein, 23 aa, Artificial Sequence
  gamma secretase cleavage
AIIGLMVGGVVIATVIVITLVML

SEQ ID NO: 48 - DNA, 69 bp, Artificial Sequence
  gamma secretase cleavage
gcaatcattggactcatggtgggcggtgttgtcatagcgacagtgatcgtcatcaccttggtgatgctg

SEQ ID NO: 49 - protein, 12 aa, Artificial Sequence
  KK
TVIVITLVMLKK

SEQ ID NO: 50 - DNA, 36 bp, Artificial Sequence
  KK
acagtgatcgtcatcaccttggtgatgctgaagaag

SEQ ID NO: 51 - DNA, 271 bp, Artificial Sequence
  human synapsin I (SYN) promoter
gcggacagtgccttcgcccccgcctggcggcgcgcgccaccgccgcctcagcactgaaggcgcgctgacgtcactcgccggtcccccgcaaactccccttcccggccaccttggtcgcgtccgcgccgccgccggcccagccggaccgcaccacgcgaggcgcgagataggggggcacgggcgcgaccatctgcgctgcggcgccggcgactcagcgctgcctcagtctgcggtgggcagcggaggagtcgtgtcgtgcctgagagcgcag

SEQ ID NO: 52 - DNA, 1293 bp, Artificial Sequence
  CamKII promoter
ttaacattatggccttaggtcacttcatctccatggggttcttcttctgattttctagaaaatgagatgggggtgcagagagcttcctcagtgacctgcccagggtcacatcagaaatgtcagagctagaacttgaactcagattactaatcttaaattccatgccttgggggcatgcaagtacgatatacagaaggagtgaactcattagggcagatgaccaatgagtttaggaaagaagagtccagggcagggtacatctacaccacccgcccagccctgggtgagtccagccacgttcacctcattatagttgcctctctccagtcctaccttgacgggaagcacaagcagaaactgggacaggagccccaggagaccaaatcttcatggtccctctgggaggatgggtggggagagctgtggcagaggcctcaggaggggccctgctgctcagtggtgacagataggggtgagaaagcagacagagtcattccgtcagcattctgggtctgtttggtacttcttctcacgctaaggtggcggtgtgatatgcacaatggctaaaaagcagggagagctggaaagaaacaaggacagagacagaggccaagtcaaccagaccaattcccagaggaagcaaagaaaccattacagagactacaagggggaagggaaggagagatgaattagcttcccctgtaaaccttagaacccagctgttgccagggcaacggggcaatacctgtctcttcagaggagatgaagttgccagggtaactacatcctgtctttctcaaggaccatcccagaatgtggcacccactagccgttaccatagcaactgcctctttgccccacttaatcccatcccgtctgttaaaagggccctatagttggaggtgggggaggtaggaagagcgatgatcacttgtggactaagtttgttcgcatccccttctccaaccccctcagtacatcaccctgggggaacagggtccacttgctcctgggcccacacagtcctgcagtattgtgtatataaggccagggcaaagaggagcaggttttaaagtgaaaggcaggcaggtgttggggaggcagttaccggggcaacgggaacagggcgtttcggaggtggttgccatggggacctggatgctgacgaaggctcgcgaggctgtgagcagccacagtgccctgctcagaagccccaagctcgtcagtcaagccggttctccgtttgcactcaggagcacgggcaggcgagtggcccctagttctgggggcagc

SEQ ID NO: 53 - DNA, 1104 bp, Artificial Sequence
  Tuba1a promoter
tccccctcaaaaaaaaggagcgctggagaaatacaagcccacacaaagagctcgtttttaaactcactcctttctccttacagtttctgaattccgtattagaagggatggctcatttctagggacaaaataacacaggctctggggtgaggtagggtcgggtaagggggcgagcggggaggggtgatgggagagcactaccgctaaagaaagcaagctctctagtaaagcgttaagtactactttgtatattgtttctcttttttcctttctctctctctctctctttgtttgtttttggtttttgagacaggatatcacactatatatccaggccgggtacaaaataaccgcagtcctccgcttcccaatgctgggatttacaggcataaaccactaagggcggttatgatgaccttgagctgcaagtcttcctgcctctgcctcccaggtgctgttgagggtcataggcgtggtctattcatactgagcttctgaattttgctcaaatattaataataatagtaataataataataaccacaataatacaactgtaaaactaaacatttacccacgcctttttgaccatcattcccatagctcttgctactttatttaaagcgaacagagatgttgaatcctgacggaacgtatttaaatttagtgtagtataaatgaaaagctggaatttaccataaagaatctcaacacaaattctgtgattaagtgttggggaaaaccttaaattatcctaactacagtttaaggtttaagctccgtataatcacccaacccccgttttctttcttccctctctacccctccccagctccaccccataatggatgctcggctagttgcttttgcgaggcctttgtctgaaggatgcaaaatctacggatgctagcgagggggggaaggggggagagattacctcataccatgtcgcttgcaccaatcaccactctcctgtcgcggcttctctgggcagacggaggggtctggaccaacaggaaaaggccttggcccatccccatggtgaccgagctgtatataaggaggcgcatccgcccaagtgccgcaggttctcttacatcgacc

SEQ ID NO: 54 - DNA, 1800 bp, Artificial Sequence
  NSE promoter
agagttttggaaagaagaacattacaagactgagctttttattcaagctggggggctcaatccatccttagctctgggttccttactgaaggaagcactcccaccccacagtaccccactcttagctctgagctcctcctctgctcgcccaatccttccaaccccctatggtggtatggctgacacagaaaatgtctgctcctgtatgggacatttgcccctcttctccaaatataagacaggatgaggcctagcttttgctgctccaaagttttaaaagaacacattgcacggcatttagggactctaaagggtggaggaggaatgagggaattgcatcatgccaaggctggtcctcatccatcactgcttccagggcccagagtggcttccaggaggtattcttacaaaggaagcccgatctgtagctaacactcagagcccattttcctgcgttaacccctcccgacctcatatacaggagtaacatgatcagtgacctgggggagctggccaaactgcgggacctgcccaagctgagggccttggtgctgctggacaacccctgtgccgatgagactgactaccgccaggaggccctggtgcagatggcacacctagagcgcctagacaaagagtactatgaggacgaggaccgggcagaagctgaggagatccgacagaggctgaaggaggaacaggagcaagaactcgacccggaccaagacatggaaccgtacctcccgccaacttagtggcacctctagcctgcagggacagtaaaggtgatggcaggaaggcagcccccggaggtcaaaggctgggcacgcgggaggagaggccagagtcagaggctgcgggtatctcagatatgaaggaaagatgagagaggctcaggaagaggtaagaaaagacacaagagaccagagaagggagaagaattagagagggaggcagaggaccgctgtctctacagacatagctggtagagactgggaggaagggatgaaccctgagcgcatgaagggaaggaggtggctggtggtatatggaggatgtagctgggccagggaaaagatcctgcactaaaaatctgaagctaaaaataacaggacacggggtggagaggcgaaaggagggcagagtgaggcagagagactgagaggcctggggatgtgggcattccggtagggcacacagttcacttgtcttctctttttccaggaggccaaagatgctgacctcaagaactcataataccccagtggggaccaccgcattcatagccctgttacaagaagtgggagatgttcctttttgtcccagactggaaatccgttacatcccgaggctcaggttctgtggtggtcatctctgtgtggcttgttctgtgggcctacctaaagtcctaagcacagctctcaagcagatccgaggcgactaagatgctagtaggggttgtctggagagaagagccgaggaggtgggctgtgatggatcagttcagctttcaaataaaaaggcgtttttatattctgtgtcgagttcgtgaacccctgtggtgggcttctccatctgtctgggttagtacctgccactatactggaataaggggacgcctgcttccctcgagttggctggacaaggttatgagcatccgtgtacttatggggttgccagcttggtcctggatcgcccgggcccttcccccacccgttcggttccccaccaccacccgcgctcgtacgtgcgtctccgcctgcagctcttgactcatcggggccccccgggtcacatgcg

SEQ ID NO: 55 - DNA, 1000 bp, Artificial Sequence
  PDGFB Promoter
gcctgcgtgtcccgaggggggtgctgggcccagtgtgagtacgtgtgactgtgactgagacagtgtgactgctgaaggcagggacacagcagctccctgactgggggcagaaggcgttaactgtgtgaaggctggttgtgggtgggtgggctctgggcctcgaacccgggggctgagggagatagtaaacagcagggtgactgacgggaagatcatgttggtagccctgcgaagatgctgcagggctgtgggggtttgtgtgactttgcagttcaacaaattcaaattcagccaacgctggcagggcctgttgtgccaggcaaccagctaggaggaggagactcggacccagcttgcagctgaagggcgctggctgccgggttctgtgggttcaccttgcggtgtcttcccttgctaacactgagtccttacaatagccccatctccaggttgaggctagatggaggggacagagggaagtgacttgcccaaggtgacccaagctcccgagtgccagggcaggatctgaattcaggctctcagactgcagagcctgagtccctccctgccatgcctgtgccagggtggaaatgtctggtcctggaggggagcgtggactcctggccttggctctggagacatccccctagaccacgtgggctcctaacctgtccatggtcactgtgctgaggggcgggacggtgggtcacccctagttcttttttccccagggccagattcatggactgaagggttgctcggctctcagagaccccctaagcgccccgccctggccccaagccctcccccagctcccgcgtcccccccctcctggcgctgactccgggccagaagaggaaaggctgtctccacccacctctcgcactctcccttctcctttataaaggccggaacagctgaaagggtggcaacttctcctcctgcagccgggagcggcctgcctgcctccctgcgcacccgcagcctcccccgctgcctc

SEQ ID NO: 56 - DNA, 1178 bp, Artificial Sequence
  EF-1alpha promoter
ggctccggtgcccgtcagtgggcagagcgcacatcgcccacagtccccgagaagttggggggaggggtcggcaattgaaccggtgcctagagaaggtggcgcggggtaaactgggaaagtgatgtcgtgtactggctccgcctttttcccgagggtgggggagaaccgtatataagtgcagtagtcgccgtgaacgttctttttcgcaacgggtttgccgccagaacacaggtaagtgccgtgtgtggttcccgcgggcctggcctctttacgggttatggcccttgcgtgccttgaattacttccactggctgcagtacgtgattcttgatcccgagcttcgggttggaagtgggtgggagagttcgaggccttgcgcttaaggagccccttcgcctcgtgcttgagttgaggcctggcctgggcgctggggccgccgcgtgcgaatctggtggcaccttcgcgcctgtctcgctgctttcgataagtctctagccatttaaaatttttgatgacctgctgcgacgctttttttctggcaagatagtcttgtaaatgcgggccaagatctgcacactggtatttcggtttttggggccgcgggcggcgacggggcccgtgcgtcccagcgcacatgttcggcgaggcggggcctgcgagcgcggccaccgagaatcggacgggggtagtctcaagctggccggcctgctctggtgcctggcctcgcgccgccgtgtatcgccccgccctgggcggcaaggctggcccggtcggcaccagttgcgtgagcggaaagatggccgcttcccggccctgctgcagggagctcaaaatggaggacgcggcgctcgggagagcgggcgggtgagtcacccacacaaaggaaaagggcctttccgtcctcagccgtcgcttcatgtgactccacggagtaccgggcgccgtccaggcacctcgattagttctcgagcttttggagtacgtcgtctttaggttggggggaggggttttatgcgatggagtttccccacactgagtgggtggagactgaagttaggccagcttggcacttgatgtaattctccttggaatttgccctttttgagtttggatcttggttcattctcaagcctcagacagtggttcaaagtttttttcttccatttcaggtgtcgtga

SEQ ID NO: 57 - DNA, 996 bp, Artificial Sequence
  CAG promoter
tgtagttaatgattaacccgccatgctacttatctacgtagccatgctctaggaagagtaccattgacgtcaataatgacgtatgttcccatagtaacgccaatagggactttccattgacgtcaatgggtggagtatttacggtaaactgcccacttggcagtacatcaagtgtatcatatgccaagtacgccccctattgacgtcaatgacggtaaatggcccgcctggcattatgcccagtacatgaccttatgggactttcctacttggcagtacatctacgtattagtcatcgctattaccatggtcgaggtgagccccacgttctgcttcactctccccatctcccccccctccccacccccaattttgtatttatttattttttaattattttgtgcagcgatgggggcggggggggggggggggcgcgcgccaggcggggcggggcggggcgaggggcggggcggggcgaggcggagaggtgcggcggcagccaatcagagcggcgcgctccgaaagtttccttttatggcgaggcggcggcggcggcggccctataaaaagcgaagcgcgcggcgggcgggagtcgctgcgcgctgccttcgccccgtgccccgctccgccgccgcctcgcgccgcccgccccggctctgactgaccgcgttactcccacaggtgagcgggcgggacggcccttctcctccgggctgtaattagcgcttggtttaatgacggcttgtttcttttctgtggctgcgtgaaagccttgaggggctccgggagggccctttgtgcggggggagcggctcggggctgtccgcggggggacggctgccttcgggggggacggggcagggcggggttcggcttctggcgtgtgaccggcggctctagagcctctgctaaccatgttcatgccttcttctttttcctacagctcctgggcaacgtgctggttattgtgctgtctcatcattttggcaaagaatt

SEQ ID NO: 58 - DNA, 508 bp, Artificial Sequence
  CMV promoter
cgttacataacttacggtaaatggcccgcctggctgaccgcccaacgacccccgcccattgacgtcaataatgacgtatgttcccatagtaacgccaatagggactttccattgacgtcaatgggtggagtatttacggtaaactgcccacttggcagtacatcaagtgtatcatatgccaagtacgccccctattgacgtcaatgacggtaaatggcccgcctggcattatgcccagtacatgaccttatgggactttcctacttggcagtacatctacgtattagtcatcgctattaccatggtgatgcggttttggcagtacatcaatgggcgtggatagcggtttgactcacggggatttccaagtctccaccccattgacgtcaatgggagtttgttttggcaccaaaatcaacgggactttccaaaatgtcgtaacaactccgccccattgacgcaaatgggcggtaggcgtgtacggtgggaggtctatataagcagagct

SEQ ID NO: 59 - protein, 18 aa, Artificial Sequence
  T2A
EGRGSLLTCGDVEENPGP

SEQ ID NO: 60 - protein, 19 aa, Artificial Sequence
  P2A
ATNFSLLKQAGDVEENPGP

SEQ ID NO: 61 - protein, 20 aa, Artificial Sequence
  E2A
QCTNYALLKLAGDVESNPGP

SEQ ID NO: 62 - protein, 22 aa, Artificial Sequence
  F2A
VKQTLNFDLLKLAGDVESNPGP

SEQ ID NO: 63 - DNA, 63 bp, Artificial Sequence
  T2A
ggctccggcgagggcaggggaagtcttctaacatgcggggacgtggaggaaaatcccggccca

SEQ ID NO: 64 - DNA, 66 bp, Artificial Sequence
  P2A
ggctccggcgccacaaacttctctctgctaaagcaagcaggtgatgttgaagaaaaccccgggcct

SEQ ID NO: 65 - DNA, 69 bp, Artificial Sequence
  E2A
ggctccggccagtgtactaattatgctctcttgaaattggctggagatgttgagagcaacccaggtccc

SEQ ID NO: 66 - DNA, 75 bp, Artificial Sequence
  F2A
ggctccggcgtgaaacagactttgaattttgaccttctcaagttggcgggagacgtggagtccaaccctggacct

SEQ ID NO: 67 - protein, 804 aa, Artificial Sequence
  Fusion protein
MLPGLALLLLAAWTARALEVPTDGNAGLLAEPQIAMFCGRLNMHMNVQNGKWDSDPSGTKTCIDTKEGILQYCQEVYPELQITNVVEANQPVTIQNWCKRGRKQCKTHPHFVIPYRCLVGEFVSDALLVPDKCKFLHQERMDVCETHLHWHTVAKETCSEKSTNLHDYGMLLPCGIDKFRGVEFVCCPLAEESDNVDSADAEEDDSDVWWGGADTDYADGSEDKVVEVAEEEEVAEVEEEEADDDEDDEDGDEVEEEAEEPYEEATERTTSIATTTTTTTESVEEVVREVCSEQAETGPCRAMISRWYFDVTEGKCAPFFYGGCGGNRNNFDTEEYCMAVCGSAMSQSLLKTTQEPLARDPVKLPTTAASTPDAVDKYLETPGDENEHAHFQKAKERLEAKHRERMSQVMREWEEAERQAKNLPKADKKAVIQHFQEKVESLEQEAANERQQLVETHMARVEAMLNDRRRLALENYITALQAVPPRPRHVFNMLKKYVRAEQKDRQHTLKHFEHVRMVDPKKAAQIRSQVMTHLRVIYERMNQSLSLLYNVPAVAEEIQDEVDELLQKEQNYSDDVLANMISEPRISYGNDALMPSLTETKTTVELLPVNGEFSLDDLQPWHSFGADSVPANTENEVEPVDARPAADRGLTTRPGSGLTNIKTEEISEVKMDAEFRHDSGYEVHHQKLPDFDEDVGSNKGAIIGLMVGGVVIATVIVITLVMLKKKQYTSIHHGVVEVDAAVTPEERHLSKMQQNGYENPTYKFFEQMQNAIIGLMVGGVVIATVIVITLVMLMDVWMINKKRK

SEQ ID NO: 68 - protein, 804 aa, Artificial Sequence
  Fusion protein
MLPGLALLLLAAWTARALEVPTDGNAGLLAEPQIAMFCGRLNMHMNVQNGKWDSDPSGTKTCIDTKEGILQYCQEVYPELQITNVVEANQPVTIQNWCKRGRKQCKTHPHFVIPYRCLVGEFVSDALLVPDKCKFLHQERMDVCETHLHWHTVAKETCSEKSTNLHDYGMLLPCGIDKFRGVEFVCCPLAEESDNVDSADAEEDDSDVWWGGADTDYADGSEDKVVEVAEEEEVAEVEEEEADDDEDDEDGDEVEEEAEEPYEEATERTTSIATTTTTTTESVEEVVREVCSEQAETGPCRAMISRWYFDVTEGKCAPFFYGGCGGNRNNFDTEEYCMAVCGSAMSQSLLKTTQEPLARDPVKLPTTAASTPDAVDKYLETPGDENEHAHFQKAKERLEAKHRERMSQVMREWEEAERQAKNLPKADKKAVIQHFQEKVESLEQEAANERQQLVETHMARVEAMLNDRRRLALENYITALQAVPPRPRHVFNMLKKYVRAEQKDRQHTLKHFEHVRMVDPKKAAQIRSQVMTHLRVIYERMNQSLSLLYNVPAVAEEIQDEVDELLQKEQNYSDDVLANMISEPRISYGNDALMPSLTETKTTVELLPVNGEFSLDDLQPWHSFGADSVPANTENEVEPVDARPAADRGLTTRPGSGLTNIKTEEISEVKMDAEFRHDSGYEVHHQKLPDFDEDVGSNKGAIIGLMVGGVVIATVIVITLVMLKKKQYTSIHHGVVEVDAAVTPEERHLSKMQQNGYENPTYKFFEQMQNAIIGLMVGGVVIATVIVITLVMLMDVQMINKKLK

SEQ ID NO: 69 - protein, 923 aa, Artificial Sequence
  Fusion protein
MLPGLALLLLAAWTARALEVPTDGNAGLLAEPQIAMFCGRLNMHMNVQNGKWDSDPSGTKTCIDTKEGILQYCQEVYPELQITNVVEANQPVTIQNWCKRGRKQCKTHPHFVIPYRCLVGEFVSDALLVPDKCKFLHQERMDVCETHLHWHTVAKETCSEKSTNLHDYGMLLPCGIDKFRGVEFVCCPLAEESDNVDSADAEEDDSDVWWGGADTDYADGSEDKVVEVAEEEEVAEVEEEEADDDEDDEDGDEVEEEAEEPYEEATERTTSIATTTTTTTESVEEVVREVCSEQAETGPCRAMISRWYFDVTEGKCAPFFYGGCGGNRNNFDTEEYCMAVCGSAMSQSLLKTTQEPLARDPVKLPTTAASTPDAVDKYLETPGDENEHAHFQKAKERLEAKHRERMSQVMREWEEAERQAKNLPKADKKAVIQHFQEKVESLEQEAANERQQLVETHMARVEAMLNDRRRLALENYITALQAVPPRPRHVFNMLKKYVRAEQKDRQHTLKHFEHVRMVDPKKAAQIRSQVMTHLRVIYERMNQSLSLLYNVPAVAEEIQDEVDELLQKEQNYSDDVLANMISEPRISYGNDALMPSLTETKTTVELLPVNGEFSLDDLQPWHSFGADSVPANTENEVEPVDARPAADRGLTTRPGSGLTNIKTEEISEVKMDAEFRHDSGYEVHHQKLPDFDEDVGSNKGAIIGLMVGGVVIATVIVITLVMLKKKQYTSIHHGVVEVDAAVTPEERHLSKMQQNGYENPTYKFFEQMQNAIIGLMVGGVVIATVIVITLVMLMQTAPVPMPDLKNVKSKIGSTENLKHQPGGGDVQPINKKLKLSNVQSKCGSKDNIKHVPGGGSVQPVYDPVDLSKVTSKCGSLGNIHHKPGGGQVEVKSEKLDFKDRVQSKIGSLDNITHVPGGGNKKIE

SEQ ID NO: 70 - protein, 65 aa, Artificial Sequence
  Fusion protein
DAEFRHDSGYEVHHQKLPDFDEDVGSNKGAIIGLMVGGVVIAAIIGLMVGGVVIATVIVITLVML

SEQ ID NO: 71 - protein, 76 aa, Artificial Sequence
  Fusion protein
DAEFRHDSGYEVHHQKLPDFDEDVGSNKGAIIGLMVGGVVIAAIIGLMVGGVVIATVIVITLVMLMDVWMINKKRK

SEQ ID NO: 72 - protein, 190 aa, Artificial Sequence
  Fusion protein
LPDFDEDVGSNKGAIIGLMVGGVVIAAIIGLMVGGVVIATVIVITLVMLMDVQMINKKLKMQTAPVPMPDLKNVKSKIGSTENLKHQPGGGDVQPINKKLKLSNVQSKCGSKDNIKHVPGGGSVQPVYDPVDLSKVTSKCGSLGNIHHKPGGGQVEVKSEKLDFKDRVQSKIGSLDNITHVPGGGNKKIE